European Patent Specification EP 3 816 293 B1, published July 19, 2023. Title: STRAINS AND PROCESSES FOR SINGLE CELL PROTEIN OR BIOMASS PRODUCTION. Applicant: Solar Foods. The sequence listing filed with the application follows.

SEQUENCE LISTING (59 sequences)

SEQ ID NO: 1 - DNA, 1482 bp, Unknown
  Novel strain
cttgagagtttgatcctggctcagagcgaacgctggcggcaggcctaacacatgcaagtcgagcgcccagcaatgggagcggcagacgggtgagtaacgcgtggggatgtgcccaatggtacggaataacccagggaaacttggactaataccgtatgagcccttcgggggaaagatttatcgccattggatcaacccgcgtctgattagctagttggtggggtaacggcccaccaaggcgacgatcagtagctggtctgagaggatgatcagccacactgggactgagacacggcccagactcctacgggaggcagcagtggggaatattggacaatgggcgcaagcctgatccagccatgccgcgtgtgtgatgaaggccttagggttgtaaagcactttcgccggtgaagataatgacggtaaccggagaagaagccccggctaacttcgtgccagcagccgcggtaatacgaagggggctagcgttgctcggaatcactgggcgtaaagcgcacgtaggcggatcgttaagtcaggggtgaaatcctggagctcaactccagaactgcccttgatactggcgaccttgagttcgagagaggttggtggaactgcgagtgtagaggtgaaattcgtagatattcgcaagaacaccagtggcgaaggcggccaactggctcgatactgacgctgaggtgcgaaagcgtggggagcaaacaggattagataccctggtagtccacgccgtaaacgatggatgctagccgttgggcagcttgctgttcagtggcgcagctaacgcattaagcatcccgcctggggagtacggtcgcaagattaaaactcaaaggaattgacgggggcccgcacaagcggtggagcatgtggtttaattcgaagcaacgcgcagaaccttaccagcctttgacatggcaggacgatttccagagatggatctcttccagcaatggacctgcacacaggtgctgcatggctgtcgtcagctcgtgtcgtgagatgttgggttaagtcccgcaacgagcgcaaccctcgcctctagttgccagcattcagttgggcactctagagggactgccggtgataagccgagaggaaggtggggatgacgtcaagtcctcatggcccttacgggctgggctacacacgtgctacaatggtggtgacagtgggatgcgaaagggcgacctctagcaaatctccaaaagccatctcagttcggattgtactctgcaactcgagtgcatgaagttggaatcgctagtaatcgtggatcagcatgccacggtgaatacgttcccgggccttgtacacaccgcccgtcacaccatgggagttggctttacccgaaggcgctgcgctaacccgcaagggaggcaggcgaccacggtagggtcagcgactggggtgaagtcgtaacaaggtagccgtaggggaacctgcggctggatcacctccttt

SEQ ID NO: 2 - DNA, 1467 bp, Unknown
  novel strain
atgggtgccgaagcaaccgtcgggcagatcacggacgccaagaagagatacgccgccggcgtgctgaagtacgcccagatgggctactggaacggcgactacgttcccaaggacaccgacctcctggcggtgttccgcatcaccccccaggcgggcgtggacccggtggaagccgccgcggcggtcgccggcgaaagctccaccgctacctggaccgtggtgtggaccgaccggctcaccgccgccgacgtctaccgcgccaaggcctacaaggtggagccggtgccgggccaggaaggccagtatttctgctacatcgcctatgatctcgatttgttcgaggaaggctccatcgccaacctcacggcgtcgatcatcggcaacgtcttctccttcaagccgctgaaggcggcgcggctggaggacatgcggcttcccgtcgcctatgtgaagaccttccgcggcccgcccaccggcatcgtggtcgagcgcgagcgcctggacaagttcggccgcccccttctgggcgccaccaccaagccgaagcttggcctctcgggcaagaattacggccgcgtggtctatgaggccctcaagggcggcctcgacttcgtgaaggacgacgagaacatcaactcgcagcccttcatgcactggcgcgatcgcttcctctattgcatggaggccgtcaacaaggcccaggccgagaccggcgaggtgaaggggcactatctcaacatcaccgccgggaccatggaggagatgtaccgccgcgccgagttcgccaaggaactgggctccgtggtggtgatggtggatctcatcatcggctggaccgccatccagtccatgtccaactggtgccgcgagaacgacatgatcctgcacatgcaccgtgcgggccatggcacctacacgcgccagaagagccacggcgtctccttccgcgtcatcgccaagtggctgcggctcgccggcgtcgaccacctgcacaccggcaccgccgtgggcaagctggaaggcgaccccatgaccgtgcagggcttctacaatgtctgccgcgagacgacgacgcagcaggacctcacccgcggcctgttcttcgagcaggactggggcggcatccgcaaggtgatgccggtggcctccggcggcatccatgcgggccagatgcaccagctcatcgacctgttcggcgaggacgtggtgctccagttcggcggcggcaccatcggccacccggacggcatccaggccggcgccaccgccaaccgcgtggcgctggaaaccatgatcctcgcccgcaacgagggccgcgacatcaggaacgagggcccggaaatcctggtggaagccgccaaatggtgccgtccgctgcgcgcggcgctcgatacctggggcgaggtgaccttcaactacgcctccaccgacacgtccgattacgtgcccaccgcgtccgtcgcctga

SEQ ID NO: 3 - protein, 488 aa, Unknown
  novel strain
MGAEATVGQITDAKKRYAAGVLKYAQMGYWNGDYVPKDTDLLAVFRITPQAGVDPVEAAAAVAGESSTATWTVVWTDRLTAADVYRAKAYKVEPVPGQEGQYFCYIAYDLDLFEEGSIANLTASIIGNVFSFKPLKAARLEDMRLPVAYVKTFRGPPTGIVVERERLDKFGRPLLGATTKPKLGLSGKNYGRVVYEALKGGLDFVKDDENINSQPFMHWRDRFLYCMEAVNKAQAETGEVKGHYLNITAGTMEEMYRRAEFAKELGSVVVMVDLIIGWTAIQSMSNWCRENDMILHMHRAGHGTYTRQKSHGVSFRVIAKWLRLAGVDHLHTGTAVGKLEGDPMTVQGFYNVCRETTTQQDLTRGLFFEQDWGGIRKVMPVASGGIHAGQMHQLIDLFGEDVVLQFGGGTIGHPDGIQAGATANRVALETMILARNEGRDIRNEGPEILVEAAKWCRPLRAALDTWGEVTFNYASTDTSDYVPTASVA

SEQ ID NO: 4 - DNA, 405 bp, Unknown
  novel strain
atgcgcatcacccaaggctccttctccttcctgccggacctcaccgacacgcagatcaaggcccaggtgcaatattgcctggaccagggctgggcggtctcggtggagcacaccgacgatccccacccgcgcaacacctattgggagatgtggggcccgcccatgttcgatctgcgcgacgcggccggcgtcttcggcgagatcgaagcctgccgggccgccaatcccgagcattatgtgcgggtgaacgccttcgattccagccgcggatgggagacgatccgcctgtccttcatcgttcagcggcccaccgtggaagagggcttccgcctcgaccgcaccgaaggcaagggccgcaaccagagctacgccatgcgctaccgggcgcagttcgcgccgcgctga

SEQ ID NO: 5 - protein, 134 aa, Unknown
  novel strain
MRITQGSFSFLPDLTDTQIKAQVQYCLDQGWAVSVEHTDDPHPRNTYWEMWGPPMFDLRDAAGVFGEIEACRAANPEHYVRVNAFDSSRGWETIRLSFIVQRPTVEEGFRLDRTEGKGRNQSYAMRYRAQFAPR

SEQ ID NO: 6 - DNA, 1896 bp, Unknown
  novel strain
atgatgccatctgagccgcacggcgcgggcatgccgcccccacgggaagcggccgcggttcccaccccccaggaggtgagcgcggtggtggccgaggtggtcgcggatgccgtggcatcggtgggcggcgcacgcacccggctcatggacatcgtccagctggcccagcagcgtctcggccatctctccgaagagaccatggcggccattgccgcgcggctcgccattccgccggtggaagtggcggacatggtgtccttctacgccttcctgaaccgcgcgcccaagggccgctaccacatccgcctgtcgcgcagccccatctcgctgatgaagggcgccgaggcggtggctgccgccttctgccagatcctcggcatcgccatgggcgagacctcgcaggatggcgacttcaccctggaatggaccaacgacatcggcatggccgaccaggagccggccgccctcgtcaacggcacggtgatgacgcagctcgcgcccggcgatgcggccatcatcgtcggccggctgcgggcccatcacgcgcccaatgccctgccgctgttccctggagccggcgtggccggctccggcctgccccatgcccggatccgccccagcctggtgatgccgggacagcttctgttccgcgaggaccacacgacgccgggcgccggcatcaaggcggcactcgccctcaccccggacgaagtggtgcagaaggtctccgccgcgcgcctgcgcgggcggggtggcgccggctttcccaccggtctcaaatggaagctctgccgccagtcgcccgccaccacccgccatgtgatctgcaatgcggacgagggcgagcccggcaccttcaaggatcgcgtgctgctcacgcaggcgccgcacctcatgttcgacggcatgaccatcgccggctacgccttgggggcgcgggagggcgtggtctatctgcgcggcgagtacgcctatctgtgggagcctctgcatgcggtcctgcgcgagcgctatgggctcgggctcgccggcgcgaacatcctgggacacgcgggcttcgacttcgacatccgcatccagctgggcgccggcgcctatatctgcggcgaggaatccgcgctggtggaatcgctggaaggcaagcgcggctcgccccgcgaccgcccccccttccccaccgtgcgcggccatctccagcagcccaccgccgtggacaatgtggagaccttcgcctgcgccgcccgcatcctggaggatggcgtggaggcgttcgcgggcatcggcacgcccgaatccgccggcacgaagctcctctcggtgtcgggcgattgcccgcgccccggcgtgtatgaggtgcccttcggcctcacggtgaacgcgctgctcgaccttgtcggcgcgccggacgccgccttcgtgcagatgggtgggccgtccggccaatgcgtggcgccgaaggattacggccgccgcatcgccttcgaggacctgcccaccggcggctcggtgatggtgttcggcccggggcgcgacgtgctcgccatggtgcgcgagttcgcggatttcttcgccggcgaatcctgcggctggtgcacgccctgccgggtgggcaccaccttgctcaaggaagagctggacaagctcctcgccaaccgcgccaccctcgccgacatccgcgcgctggagaccctggccacgaccgtctcccgcaccagccgctgcggcctcggccagacggcgcccaaccccatcctttccaccatgcgcaacctgccggaagcctatgaggcgaggctgaggcccgaagacttcctgccctgggcctcgctcgacgaggcgctgaagcccgccatcgtcatccagggccgcgcgcccgtgccggaggaagaggcatga

SEQ ID NO: 7 - protein, 631 aa, Unknown
  novel strain
MMPSEPHGAGMPPPREAAAVPTPQEVSAVVAEVVADAVASVGGARTRLMDIVQLAQQRLGHLSEETMAAIAARLAIPPVEVADMVSFYAFLNRAPKGRYHIRLSRSPISLMKGAEAVAAAFCQILGIAMGETSQDGDFTLEWTNDIGMADQEPAALVNGTVMTQLAPGDAAIIVGRLRAHHAPNALPLFPGAGVAGSGLPHARIRPSLVMPGQLLFREDHTTPGAGIKAALALTPDEVVQKVSAARLRGRGGAGFPTGLKWKLCRQSPATTRHVICNADEGEPGTFKDRVLLTQAPHLMFDGMTIAGYALGAREGVVYLRGEYAYLWEPLHAVLRERYGLGLAGANILGHAGFDFDIRIQLGAGAYICGEESALVESLEGKRGSPRDRPPFPTVRGHLQQPTAVDNVETFACAARILEDGVEAFAGIGTPESAGTKLLSVSGDCPRPGVYEVPFGLTVNALLDLVGAPDAAFVQMGGPSGQCVAPKDYGRRIAFEDLPTGGSVMVFGPGRDVLAMVREFADFFAGESCGWCTPCRVGTTLLKEELDKLLANRATLADIRALETLATTVSRTSRCGLGQTAPNPILSTMRNLPEAYEARLRPEDFLPWASLDEALKPAIVIQGRAPVPEEEA

SEQ ID NO: 8 - DNA, 1491 bp, Unknown
  novel strain
atgagccggggatcccccgatgccgggaaagaccgcaccatgagcgccaccgacggcaccaccgccccccgcaagatcgtcatcgatccggtgacccgcgtggagggccacggcaaggtcaccatccgcctggatgaagccggcgcggtggaggatgcgcgtttccacatcgtggagttccgcggcttcgagcggttcatccagggccggatgtactgggaagtgccccttatcatccagcggctgtgcggcatctgcccggtgagccaccatctggcggcggcgaaagccatggaccaggtggcgggcgtggaccgcgtaccgcccaccgccgagaaactgcgccggctgatgcattatgggcaggtgctgcaatccaacgctttgcacatcttccacctcgcctcgcccgacctcctgttcggcttcgacgcgccggccgagcagcgcaacatcatcgccgtgctccagcgttatccggagatcggcaaatgggcgatcttcatcaggaagttcggccaggaggtcatcaaggccaccggcgggcgcaagatccatcccaccagcgccattcccggcggggtcaaccagaacctcgccgtggaggaccgcgacgccctgcgcgccaaggtgggcgagatcatcagctggtgcatggcggcgctggaccatcacaaggcctatgtggcggaaaaccgggcgctgcatgacagcttcgccgccttcccctccgccttcatgagcctcgtggggccggatggcggcatggacctttatgacggcaccctgcgggtgatcgatgccgagggcgcccccctcatcgaaggcgcgccgcccgcctcctaccgcgaccacctcatcgaggaggtgcggccctggagctatctgaaattcccccatctgcgcgccttcggccgcgacgatggctggtatcgggtcggccccctcgcccaggtcaattgcgccgcgtccatcgacacgccccgcgccgaggcggcccggcgggacttcatggccgagggcggcggcaagccggtgcatgccaccctcgcttatcactgggcgcggctcatcgtgctggtccattgcgcggagaagatcgaacagctgctgttcgacgacgacctgcaaggctgcgatctgcgtgcggagggcacccggcgcggggaaggcgtcgcctggatcgaggcgccgcgcggcaccctcatccaccattacgaggtggacgagaacgaccaggtgcgccgcgccaacctcatcgtctccaccacccacaataacgaggccatgaaccgcgccgtgcggcaggtggcgaagacggacctttccggtcgcgagatcaccgaagggctgctgaaccatatcgaggtggccatccgcgccttcgacccctgcctgtcctgcgccacccatgcgctgggccagatgccgctgatcgtgacgcttgaagatgcctccggcgcagagatcgcccgcggagtgaaggaatga

SEQ ID NO: 9 - protein, 496 aa, Unknown
  novel strain
MSRGSPDAGKDRTMSATDGTTAPRKIVIDPVTRVEGHGKVTIRLDEAGAVEDARFHIVEFRGFERFIQGRMYWEVPLIIQRLCGICPVSHHLAAAKAMDQVAGVDRVPPTAEKLRRLMHYGQVLQSNALHIFHLASPDLLFGFDAPAEQRNIIAVLQRYPEIGKWAIFIRKFGQEVIKATGGRKIHPTSAIPGGVNQNLAVEDRDALRAKVGEIISWCMAALDHHKAYVAENRALHDSFAAFPSAFMSLVGPDGGMDLYDGTLRVIDAEGAPLIEGAPPASYRDHLIEEVRPWSYLKFPHLRAFGRDDGWYRVGPLAQVNCAASIDTPRAEAARRDFMAEGGGKPVHATLAYHWARLIVLVHCAEKIEQLLFDDDLQGCDLRAEGTRRGEGVAWIEAPRGTLIHHYEVDENDQVRRANLIVSTTHNNEAMNRAVRQVAKTDLSGREITEGLLNHIEVAIRAFDPCLSCATHALGQMPLIVTLEDASGAEIARGVKE

SEQ ID NO: 10 - DNA, 720 bp, Unknown
  novel strain
atgagcgagacccccttcacctttaccgtggacggcatcgcggtcccggccacccccggccagagcgtcatcgaggcgtgcgatgcggcgggcatctatatcccgcgcctgtgccaccacccggacctgccgccggcgggccattgccgggtgtgcacctgcatcatcgacgggcggccggccagcgcctgcaccatgcccgccgccaggggcatggtggtggagaacgagacgcccgctttgctggcggagcggcgcacgctgatcgagatgctgttcgcggaaggcaaccatttctgccagttctgcgaggcgagcggcgattgcgaattgcaggcgctgggctacctgttcggcatggtggccccgcccttcccccatctgtggccgaagcggccggtggatgccagccatccggatatctatatcgaccacaatcgctgcatcctgtgctcgcgctgcgtgcgcgcctcgcgcaccctggacggcaagtccgtgttcggcttcgaggggcgcggcatcgagatgcatctggcggtgaccggcgggcacctggacgacagcgccatcgccgccgccgacagggcggttgagatgtgcccggtgggctgcatcgtcctcaagcgcaccggctaccgcacgccctatggccggcggcgctacgacgccgcgcccatcggctccgacatcaccgcccggcgcggcggcgcgaaggactga

SEQ ID NO: 11 - protein, 239 aa, Unknown
  novel strain
MSETPFTFTVDGIAVPATPGQSVIEACDAAGIYIPRLCHHPDLPPAGHCRVCTCIIDGRPASACTMPAARGMVVENETPALLAERRTLIEMLFAEGNHFCQFCEASGDCELQALGYLFGMVAPPFPHLWPKRPVDASHPDIYIDHNRCILCSRCVRASRTLDGKSVFGFEGRGIEMHLAVTGGHLDDSAIAAADRAVEMCPVGCIVLKRTGYRTPYGRRRYDAAPIGSDITARRGGAKD

SEQ ID NO: 12 - DNA, 543 bp, Unknown
  novel strain
atggccaagcccaaactcgccacctgcgcgctggccggctgcttcggctgccacatgtccttcctggacatggacgagcgcatcgtcgagctcatcgacctggtggacctcgacgtctcgcccctcgacgacaagaaaaacttcaccggcatggtggaaatcggcctggtggaaggcggctgcgccgacgagcgccatgtgaaggtgctgcgcgagttccgcgagaaatcccgcatcctggtggcggtgggcgcctgcgccatcaccggcggcatcccggcattgcgcaacctcgccggcctcgacgaatgcctgagggaagcctacctcaccggccccacggtggaaggcggcgggctcattcccaacgacccggagctgccgctgctgctggacaaggtctatccggtgcaggacttcgtgaagatcgaccatttcctgcccggctgcccgccctcggccgacgccatctgggcggctctgaaggcgctgctgaccggcaccgagccgcatctgccctacccgcttttcaagtacgaatga

SEQ ID NO: 13 - protein, 180 aa, Unknown
  novel strain
MAKPKLATCALAGCFGCHMSFLDMDERIVELIDLVDLDVSPLDDKKNFTGMVEIGLVEGGCADERHVKVLREFREKSRILVAVGACAITGGIPALRNLAGLDECLREAYLTGPTVEGGGLIPNDPELPLLLDKVYPVQDFVKIDHFLPGCPPSADAIWAALKALLTGTEPHLPYPLFKYE

SEQ ID NO: 14 - DNA, 1013 bp, Unknown
  novel strain
tccagacccgggcaacattgctccatgtgctgggcaccctggccggccgctggccccataccctcgcgctccagcccggcggggtgacccgaagcgccgaccagcacgaccgcatgcgcctgctcgcgacgctgaaggcggtgcgggcggcgctggaagagaccttgttcggcgcgcctttggaagaggtggcggccctggacggcgccgccgccgtggaggcctggcgcgccaacggcccggaaggggatttccgcctgttcctggagatcgccgccgacctggagctggaccggctcggccgcgcgcacgaccgctttctctccttcggcgcctacgcccaggacgaggggcgcctttatggcgccggcaccttcgaggccgggacggcgggagggctcgatcccaacgccatcaccgaggaccacgccttcgcccgcatggaggaccgcgcggcgccccatgcgccctttgacggctccaccttccccgatgccgacgacaccgagggctacacctggtgcaaggcgccgcgccttgccggcctgcccttcgagaccggcgccttcgcccggcaggtggtggcgggccatccgctcgcccgggacctcgtgacgcgggaaggcggcactgtgcgcagccgcgtggtcggccggctgctggaaaccgcgcgcaccctgatcgccatggagggctgggtgaaggaactgcggcccgaagggccctggtgcgcccagggccacctgccccaggaaggccgcgccttcggcctcaccgaggcggcgcgcggggcgctcggccactggatggtggtggagaagggccgcattgcccgctaccagatcatcgcccccaccacctggaacttctccccccgcgacggcgcgggcctgcccggcccgctggagacggccctggtgggcgcgcccgtgcggcagggagagacgacgcccgtgagcgtgcagcacatcgtgcgctccttcgacccgtgcatggtctgcactgtgcattga

SEQ ID NO: 15 - protein, 485 aa, Unknown
  novel strain
MSAETRRLVVGPFNRVEGDLEVRLDVQDGRVQQAFVSSPLFRGFERILEGRDPRDALVIAPRICGICSVSQSHAAALALAGLQGIAPTHDGRIATNLIVAAENVADHLTHFHVFFMPDFARAVYEDRPWFAQAARRFKANQGVSVRRALQTRATLLHVLGTLAGRWPHTLALQPGGVTRSADQHDRMRLLATLKAVRAALEETLFGAPLEEVAALDGAAAVEAWRANGPEGDFRLFLEIAADLELDRLGRAHDRFLSFGAYAQDEGRLYGAGTFEAGTAGGLDPNAITEDHAFARMEDRAAPHAPFDGSTFPDADDTEGYTWCKAPRLAGLPFETGAFARQVVAGHPLARDLVTREGGTVRSRVVGRLLETARTLIAMEGWVKELRPEGPWCAQGHLPQEGRAFGLTEAARGALGHWMVVEKGRIARYQIIAPTTWNFSPRDGAGLPGPLETALVGAPVRQGETTPVSVQHIVRSFDPCMVCTVH

SEQ ID NO: 16 - DNA, 858 bp, Unknown
  novel strain
acgggggaggaagcccgcgccatcttcgacgccatccttgccggcgttatcgtcctcgacgccctgtgcgtggaaggcgcgctgctgcgcgggccgaacggcaccgggcgcttccatgtgctggcgggcacggacacccccaccatcgactgggcgcggcagctcgccggcatggcgcgccacgtggtggcggtgggcacctgcgccgcctatgggggcgtgacggcggcgggcatcaaccccaccgatgcctgcggcctccagttcgacggacgccggaagggtggggcgctgggggcggacttccgctcccgctcggggcttccggtcatcaatgtggccggctgccccacccatcccaactgggtgacggaaaccctgatgctgctcgcctgcggcctgctgggcgaggccgacctcgacgtctatggccgcccgcgcttctatgcggacctgctggtgcatcacggctgcccgcgcaacgaatactatgaatacaaggcgagcgccgagaagatgagcgacctcggctgcatgatggagcatctgggctgcctcggcacccaggcccacgccgactgcaacacgcgcctttggaatggcgagggctcgtgcacccgcggcggctatgcctgcatcaactgcacggcgccggaattcgaggagccgggccacgccttcctggagacgcccaagatcggcggcatccccatcggcctgcccaccgacatgcccaaggcctggttcatcgccttgtcctccctcgccaaggcggcgacgccggagcggctgcgcaagaacgcggtgtccgaccatgtggtcacgccgcccgccgtcaaggacatcaagcggcgatga

SEQ ID NO: 17 - protein, 335 aa, Unknown
  novel strain
MSTPFSVLWLQSGGCGGCTMSLLCAEAPDLATTLDAAGIGFLWHPALSEETGEEARAIFDAILAGVIVLDALCVEGALLRGPNGTGRFHVLAGTDTPTIDWARQLAGMARHVVAVGTCAAYGGVTAAGINPTDACGLQFDGRRKGGALGADFRSRSGLPVINVAGCPTHPNWVTETLMLLACGLLGEADLDVYGRPRFYADLLVHHGCPRNEYYEYKASAEKMSDLGCMMEHLGCLGTQAHADCNTRLWNGEGSCTRGGYACINCTAPEFEEPGHAFLETPKIGGIPIGLPTDMPKAWFIALSSLAKAATPERLRKNAVSDHVVTPPAVKDIKRR

SEQ ID NO: 18 - DNA, 870 bp, Unknown
  novel strain
gtgaccgagcgcctgtccgacgtcaacgcccgcatcgcctcggtgcggcagctctcatcggtcatcacggccatgcggggcattgcggcggcgcgggcgcgggaggcgcggggtcggctcgacggcatccgcgcctatgcgcagaccatcgccgaggccatcggccatgtgctcgccgtgctgcccgaggaggcccgcgcccggtcctccgggcaccggcatcggggccatgcggtcatcgccctgtgcgcggagcagggctttgccggcgtcttcaacgagcgggtgctggacgaggccgcccggctgctgaccggcggggcggggccggccgagctgctgctggtgggcgaccggggcctgatggtggcccgcgagcgggggctcgatgtctcctggtcggtgcccatggtggcccatgcgggccaggcctcggcgctggcggaccgcatcagcgaggagctctaccggcggatcgatgcgggacgggtgacgcgggtgtcggtggtgcacgccgagcccgccgcgtccgccgccatcgagacggtggtgaaagtgctggtgccgttcgacttcgcccgcttccccctggcgcgggtggcatccgccccgctcatgaccatgccgccgccgcggctgctggcccagctgtcggaggaatatgtgttcgccgagctgtgcgaggcgctcaccttgtccttcgcggcggagaacgaggcccgcatgcgggccatgatcgccgcccgcgccaatgtggccgataccctggagggcctcgtcggccgcgcccggcagatgcgccaggaggagatcaccaacgagatcatcgagctggaaggcggcgccggcagcgcccggcatgcggattga

SEQ ID NO: 19 - protein, 289 aa, Unknown
  novel strain
MTERLSDVNARIASVRQLSSVITAMRGIAAARAREARGRLDGIRAYAQTIAEAIGHVLAVLPEEARARSSGHRHRGHAVIALCAEQGFAGVFNERVLDEAARLLTGGAGPAELLLVGDRGLMVARERGLDVSWSVPMVAHAGQASALADRISEELYRRIDAGRVTRVSVVHAEPAASAAIETVVKVLVPFDFARFPLARVASAPLMTMPPPRLLAQLSEEYVFAELCEALTLSFAAENEARMRAMIAARANVADTLEGLVGRARQMRQEEITNEIIELEGGAGSARHAD

SEQ ID NO: 20 - DNA, 1536 bp, Unknown
  novel strain
atgagcacgggcgcgcaagcgagcgaggattggctcacccggagccgggcggccctggccgggacgcgcctttcccagcaatcccaatcggtgggccgggtggaggagatggccgacggcatcgcccgcgtctccggcctgccggatgtgcggctcgacgagcttctcaccttcgagggcggccagaccggctatgccctcaccctcgatcgcaccgagatcgccgtggtgctgctggatgacgcctccggcgtggaggcgggcgcccgggtgttcggcaccggcgaggtggtgaaggtgccggtggggccggggctgctgggccgcatcgtcgaccccctcggccggcccatggaccgctccgagccggtggtggcgcaggcgcaccatcccatcgagcggccggcgccggccatcatcgcccgcgacctggtctcgcagccggttcagaccggcacgctggtggtggatgcgctgttctccctcggccggggccagcgcgagctcatcatcggcgaccgggctaccggcaagaccgccatcgcggtggacaccatcatcagccagaagcattcggacatcgtgtgcatctacgtggcggtgggccagcgcgccgccgccgtggagcgggtggtggaggcggtgcgcgcccacggggcgatcgagcgctgcatcttcgtggtcgcctcggccgccgcctcgccagggctgcaatggatcgcgccgttcgccggcatgaccatggcggaatatttccgcgacaacggccagcatgcgctcatcatcatcgatgatctcaccaagcatgcggccacccatcgcgagctggcgctgctcacccacgagccgccgggccgcgaggcctatcccggcgacatcttctatgtgcacgcccgccttctggagcgggccgccaagctctccgccgagctgggcggtggctcgctcacggccctgcccatcgcggagacggacgcgggaaacctctccgcctatatccccaccaacctcatctccatcaccgatgggcagatcgtgctggattcgcggctgttcgcggccaaccagcgcccggcggtggatgtgggcctctccgtgagccgggtgggcggcaaggcgcagcatcccgcgcttcgggccgtgtccgggcgcatccggctcgattattcccagttcctggagctggaaatgttcacccgcttcggcggcatcaccgatacccgcgtgaaggcgcagatcacccggggcgagcgcatccgcgcgctgctcacccagccgcgcttttccaccctgcgccttcaggacgaggtggcgctgctggccgcgctggcggagggggtgttcgacactttggccccggggctgatgggcgccgtgcgtgcccgcattccggcccagctggatgcgcaggtgaaggacgtggcctcggccctcgccgagggcaaggtgctggaggagggcttgcacgcccgtctcgtggcggccgtgcgggccgtcgcggcggacgtggccgcgaccgcgaaggccgggccgtga

SEQ ID NO: 21 - protein, 511 aa, Unknown
  novel strain
MSTGAQASEDWLTRSRAALAGTRLSQQSQSVGRVEEMADGIARVSGLPDVRLDELLTFEGGQTGYALTLDRTEIAVVLLDDASGVEAGARVFGTGEVVKVPVGPGLLGRIVDPLGRPMDRSEPVVAQAHHPIERPAPAIIARDLVSQPVQTGTLVVDALFSLGRGQRELIIGDRATGKTAIAVDTIISQKHSDIVCIYVAVGQRAAAVERVVEAVRAHGAIERCIFVVASAAASPGLQWIAPFAGMTMAEYFRDNGQHALIIIDDLTKHAATHRELALLTHEPPGREAYPGDIFYVHARLLERAAKLSAELGGGSLTALPIAETDAGNLSAYIPTNLISITDGQIVLDSRLFAANQRPAVDVGLSVSRVGGKAQHPALRAVSGRIRLDYSQFLELEMFTRFGGITDTRVKAQITRGERIRALLTQPRFSTLRLQDEVALLAALAEGVFDTLAPGLMGAVRARIPAQLDAQVKDVASALAEGKVLEEGLHARLVAAVRAVAADVAATAKAGP

SEQ ID NO: 22 - DNA, 741 bp, Unknown
  novel strain
atgcagatcgactggtggacgctgggcctgcagacggtcaacgtcctcgttctcatctggctcctgagccgcttcctgttcaagccggtggcgcaggtcatcgcgcagcgccgtgccgagatcgagaagctggtggaggatgcgcgcgccgccaaggccgccgccgaggccgagcgggacacggcgaaggcggaggaggcgcgccttgccgccgagcgcggcgcccgcatggcggcggtcgccaaggaggcggaggcgcagaaggcggcattgctggccgccgccaagaccgaggccgaggccctgcacgcggccgcggaagcggccatcgtccgggcgcgggcgagcgaggaggaagccgccgccgaccgcgccagccgccttgccgtggacatcgccgccaagctgctggaccggctgcccgacgacgcccgggtcgcgggcttcatcgatggcctcgccgaggggcttgaagccctgcccgaggcgagccgggcggtgatcggcgtcgacggcgcgccagtgcgcgtgacggccgcgcgcgcccttatgccggcggaggaggaggcctgccgcacgcggctctcccaggcgctgggccgtccggtgacgctggccgtgaccatcgaccccgccctcatcgccggcctggagatggagacgccccacgcggtggtgcgcaattccttcaaggccgatctcgaccgcgtcaccgcggcgctcacccatcatgggacctga

SEQ ID NO: 23 - protein, 246 aa, Unknown
  novel strain
MQIDWWTLGLQTVNVLVLIWLLSRFLFKPVAQVIAQRRAEIEKLVEDARAAKAAAEAERDTAKAEEARLAAERGARMAAVAKEAEAQKAALLAAAKTEAEALHAAAEAAIVRARASEEEAAADRASRLAVDIAAKLLDRLPDDARVAGFIDGLAEGLEALPEASRAVIGVDGAPVRVTAARALMPAEEEACRTRLSQALGRPVTLAVTIDPALIAGLEMETPHAVVRNSFKADLDRVTAALTHHGT

SEQ ID NO: 24 - DNA, 243 bp, Unknown
  novel strain
atgactgtcgagatggtcagcatcttcgcggcggcgctcgccgtctccttcggcgccatcgggccggccctgggcgagggccgggcggtggccgcggccatggacgccatcgcccgccagccggaggcggccggaaccttgtcgcgcacgctcttcgtcggcctcgccatgatcgagaccatggcgatctactgcctggtgatcgcgctcctggtgctcttcgccaatccgttcgtgaagtga

SEQ ID NO: 25 - protein, 80 aa, Unknown
  novel strain
MTVEMVSIFAAALAVSFGAIGPALGEGRAVAAAMDAIARQPEAAGTLSRTLFVGLAMIETMAIYCLVIALLVLFANPFVK

SEQ ID NO: 26 - DNA, 699 bp, Unknown
  novel strain
atgggctcgccgctgatcctcgaacccctgttccatatcgggcccgtgcccatcaccgcgccggtggtggtcacctggctcatcatggccgccttcattgggctggcgcggctcatcacccggaagctttccaccgatcccacccggacccaggcggcggtggaaacggtgctgaccgccatcgattcccagatcgccgacaccatgcaggccgatcccgcgccttatcgcgcgctcatcggcaccatcttcctttatgtgctggtggccaactggtcctcgctcatcccgggcatcgagccgcccacggcgcatatcgagaccgatgcggcgctcgctttcatcgtgttcgccgccaccatcgggttcgggttgaagacaaggggtgtgaagggctatctcgccaccttcgccgaaccctcctgggtgatgatcccgctcaatgtggtggagcagatcacccggaccttctcgctcatcgtgcgcctgttcggcaacatcatgagcggggtgttcgtggtcggcatcatcctgtccctcgccgggctgctggtgcccatccccctcatggcgctcgatctcctgaccggcgccgtgcaggcctacatcttcgcggtgctggcctgcgtgttcatcggcgcggccattggcgaggcgccggcaaagccccaatcgaaggagccagggaaaacatcatga

SEQ ID NO: 27 - protein, 232 aa, Unknown
  novel strain
MGSPLILEPLFHIGPVPITAPVVVTWLIMAAFIGLARLITRKLSTDPTRTQAAVETVLTAIDSQIADTMQADPAPYRALIGTIFLYVLVANWSSLIPGIEPPTAHIETDAALAFIVFAATIGFGLKTRGVKGYLATFAEPSWVMIPLNVVEQITRTFSLIVRLFGNIMSGVFVVGIILSLAGLLVPIPLMALDLLTGAVQAYIFAVLACVFIGAAIGEAPAKPQSKEPGKTS

SEQ ID NO: 28 - DNA, 456 bp, Unknown
  novel strain
gtgagcgcgccgctgcacctcaccatcaccacgccggccgccgttctggtggaccgtgccgacatcgtggccctgcgtgccgaggacgagagcggcagcttcggcatcctgcccggccatgcggatttcctgaccgttctggaggcctgcgtggtgcgcttcaaggatggggccgacggcgtgcattattgtgctctcagtggtggcgtgctgtcggtcgaggagggccggcgcatcgccatcgcctgccgtcagggcacggtgagcgacgacctggtcgccctggaaggggcggtggacgccatgcgttcggcggagagcgatgccgacaagcgggcccgggtggagcagatgcgccttcatgcccacgccgtgcgccagctcctgcactatctgcggcccggccgggccggcggcgtggcgccggccgccgcgccggaggaggggccgtcatga

SEQ ID NO: 29 - protein, 151 aa, Unknown
  novel strain
MSAPLHLTITTPAAVLVDRADIVALRAEDESGSFGILPGHADFLTVLEACVVRFKDGADGVHYCALSGGVLSVEEGRRIAIACRQGTVSDDLVALEGAVDAMRSAESDADKRARVEQMRLHAHAVRQLLHYLRPGRAGGVAPAAAPEEGPS

SEQ ID NO: 30 - DNA, 1494 bp, Unknown
  novel strain
atggcagcggcagatgaggaggcgcaatcggccgccggccccgcctcgggccgggtggtggccgtgcgcggcgcggtgatcgacatcgcctttgcccagcctccgctgccgccgctggacgacgcccttctcatcaccgacggccggggcggcacggtgctggtggaggtgcagagccatatggatcggcacacggtgcgcgccatcgcccttcaggccaccaccggcctcagccgggggctggaggcggcgcgggtgggcgggccggtgaaggtgccggtgggagaccatgtgctcggccgcctcctggatgtcaccggcgccatcggcgacaagggcgggccgctgccggccgacgtgcccacgcggccgatccaccacgcgccgccatccttcgccgcgcagggcggcacgtccgatctgtttcgcaccggcatcaaggtcatcgacctcctggcgcccctcgcccagggcggcaaggcggccatgttcggcggggccggcgtgggcaagaccgtgctggtgatggagctgatccacgccatggtggcgagctacaagggcatctcggtgtttgccggcgtgggggagcgctcccgcgagggccacgagatgctgctggacatgaccgattccggcgtgctcgaccgcaccgttctggtctatggccagatgaacgagccccccggggcccgctggcgggtgcccatgacggcgctgaccatcgccgaatatttccgcgacgagaagcaccagaacgtcctgctgctgatggacaacatcttccgcttcgtccaggcgggggcggaggtctccggccttttgggccgtccgccctcccgggtgggataccagccgacgctggcgagcgaggtggcggcgctccaggaacgcatcacctccgtgggcgaggcctcggtgaccgccatcgaggcggtctacgtgccggcggatgacttcaccgatcccgccgtgaccaccatcgccgcccacgtggattccatggtggtgctctcccgcgccatggcggcggagggcatgtatccggcggtggaccccatctcctcctcgtcggtgctgctcgacccgctcatcgtgggggacgagcatgcgcgcgtcgccaacgaggtgcgccggaccatcgagcattatcgcgagcttcaggatgtgatctcgctgctgggcatggaggaattgggcaccgaggatcgccgcatcgtggagcgggcgcgccggctccagcgcttcctcacccagcccttcacggtcaccgaggccttcaccggcgtgcccggccgctcggtggccatcgccgacaccatcgccggctgcaggatgatcctgtccggcgcctgcgacgactggcaggaaagcgccctctacatggtgggcaccatcgacgaggcccgccagaaggaggaggccgctcgcgccaaggcggggcagggcgccccggccgggacggcagccgagacggcggaggccgccccgtga

SEQ ID NO: 31 - protein, 497 aa, Unknown
  novel strain
MAAADEEAQSAAGPASGRVVAVRGAVIDIAFAQPPLPPLDDALLITDGRGGTVLVEVQSHMDRHTVRAIALQATTGLSRGLEAARVGGPVKVPVGDHVLGRLLDVTGAIGDKGGPLPADVPTRPIHHAPPSFAAQGGTSDLFRTGIKVIDLLAPLAQGGKAAMFGGAGVGKTVLVMELIHAMVASYKGISVFAGVGERSREGHEMLLDMTDSGVLDRTVLVYGQMNEPPGARWRVPMTALTIAEYFRDEKHQNVLLLMDNIFRFVQAGAEVSGLLGRPPSRVGYQPTLASEVAALQERITSVGEASVTAIEAVYVPADDFTDPAVTTIAAHVDSMVVLSRAMAAEGMYPAVDPISSSSVLLDPLIVGDEHARVANEVRRTIEHYRELQDVISLLGMEELGTEDRRIVERARRLQRFLTQPFTVTEAFTGVPGRSVAIADTIAGCRMILSGACDDWQESALYMVGTIDEARQKEEAARAKAGQGAPAGTAAETAEAAP

SEQ ID NO: 32 - DNA, 1437 bp, Unknown
  novel strain
atggcgaacaaggtcggacgcatcacccagatcatcggcgccgtcgtcgacgtgcagttcgacgggcatctgccggcgattctcaacgcgatcgagaccaccaaccagggcaaccggctggtgctcgaagtggctcagcatctcggcgagaacaccgtgcgctgcatcgccatggatgccactgaaggcctggtgcgtggccaggaggtggccgacaccgatgcgcccatccaggtgcccgtgggcgccgccaccctcggccgcatcatgaacgtgatcggcgagccggtggacgagctgggccccatcgagggcgaagcgctgcgcggcatccatcagccggccccctcctatgcggagcaggccacggaagctgagatcctcgtcaccggcatcaaggtggtggatctgctggcgccctattccaagggcggcaaggtgggcctgttcggcggcgccggcgtgggcaagaccgtgctcatcatggagctgatcaacaacgtggccaaggcgcacggcggctattccgtgttcgccggcgtgggtgagcgcacccgcgagggcaacgacctctaccacgagatgatcgagtccaacgtgaacaaggacccgcacgagaacaatggctcggcggccggttccaagtgcgccctggtctatggccagatgaacgagccgcccggcgcccgcgcccgcgtggccctcaccggcctcaccgtcgccgagcatttccgcgaccagggccaggacgtgctgttcttcgtggacaacatcttccgcttcacccaggcgggctccgaggtgtcggcgcttctcggccgcatcccctcggcggtgggctaccagccgacgctggccaccgacatgggccagctgcaggagcgcatcaccaccaccaccaagggctccatcacctcggtgcaggccatctacgtgccggcggacgatctgaccgatccggcgccggccgcctccttcgcccatctggacgccaccacggtgctgtcgcgctccatcgcggagaagggcatctacccggcggtggatccgctggactccacctcgcgcatgctgtctcccgccatcctcggcgacgagcactacaacaccgcgcgccaggtgcagcagaccctgcagcgctacaaggcgctccaggacatcatcgccatcctgggcatggacgaactctccgaagaggacaagctcaccgtggcccgcgcccgcaagatcgagcgcttcctctcccagcccttccacgtggccgaggtgttcaccggttcgcccggcaagctggtcgacctcgccgacaccatcaagggcttcaagggcctggtggacggcaagtacgactacctgcccgagcaggccttctacatggtgggcaccatcgaagaagccatcgagaagggcaagaagctggcggccgaggcggcctga

SEQ ID NO: 33 - protein, 478 aa, Unknown
  novel strain
MANKVGRITQIIGAVVDVQFDGHLPAILNAIETTNQGNRLVLEVAQHLGENTVRCIAMDATEGLVRGQEVADTDAPIQVPVGAATLGRIMNVIGEPVDELGPIEGEALRGIHQPAPSYAEQATEAEILVTGIKVVDLLAPYSKGGKVGLFGGAGVGKTVLIMELINNVAKAHGGYSVFAGVGERTREGNDLYHEMIESNVNKDPHENNGSAAGSKCALVYGQMNEPPGARARVALTGLTVAEHFRDQGQDVLFFVDNIFRFTQAGSEVSALLGRIPSAVGYQPTLATDMGQLQERITTTTKGSITSVQAIYVPADDLTDPAPAASFAHLDATTVLSRSIAEKGIYPAVDPLDSTSRMLSPAILGDEHYNTARQVQQTLQRYKALQDIIAILGMDELSEEDKLTVARARKIERFLSQPFHVAEVFTGSPGKLVDLADTIKGFKGLVDGKYDYLPEQAFYMVGTIEEAIEKGKKLAAEAA

SEQ ID NO: 34 - DNA, 876 bp, Unknown
  novel strain
atggcgagtctgaaggacctgagaaaccgcattgcctcggtgaaggcgacgcagaagatcaccaaggcgatgcagatggtcgccgcggcgaagctgcgtcgcgcccaggcggcggctgaagcggcccgtccctatgcggaacgcatggagacggtgctcggaaatcttgcctccggcatggtggtgggcgcgcaggcgcctgttctcatgaccgggacgggcaagagcgacacccacctgctgctggtgtgcaccggcgagcgcggcctgtgcggcgccttcaactcgtccatcgtgcgcttcgcccgcgagcgggcgcagctgctgctggccgagggcaagaaggtgaaaatcctgtgcgtgggccgcaagggccacgagcagctgcgccgcatctacccggacaacatcatcgacgtggtggacctgcgcgcggtgcgcaacatcggcttcaaggaggccgacgccatcgcccgcaaggtgctggccctgctcgatgaaggcgcattcgacgtctgcacgctcttctactcccacttcaggagcgtgatcgcccaggtgccgacggcccagcagctcattccggccaccttcgacgagcggccggccgtcgccgatgcgccggtctatgaatatgagccggaggaggaggagatcctcgccgagctgctgccgcgcaacgtggcggtgcagatcttcaaggccctcctcgagaaccaggcttctttctatggctcccagatgagcgccatggacaacgccacgcgcaatgcgggcgagatgatcaagaagcagacgctcacctacaaccgtacccgccaggccatgatcacgaaggaactcatcgagatcatctccggcgccgaggccgtctga

SEQ ID NO: 35 - protein, 291 aa, Unknown
  novel strain
MASLKDLRNRIASVKATQKITKAMQMVAAAKLRRAQAAAEAARPYAERMETVLGNLASGMVVGAQAPVLMTGTGKSDTHLLLVCTGERGLCGAFNSSIVRFARERAQLLLAEGKKVKILCVGRKGHEQLRRIYPDNIIDVVDLRAVRNIGFKEADAIARKVLALLDEGAFDVCTLFYSHFRSVIAQVPTAQQLIPATFDERPAVADAPVYEYEPEEEEILAELLPRNVAVQIFKALLENQASFYGSQMSAMDNATRNAGEMIKKQTLTYNRTRQAMITKELIEIISGAEAV

SEQ ID NO: 36 - DNA, 1530 bp, Unknown
  novel strain
atggacattcgagccgctgaaatctctgccatcctgaaagagcagatccagaatttcggccaggaggcggaagtctccgaggtgggtcaggttctgtccgtgggtgacggcatcgcgcgcgtctacggcctcgacaacgtccaggcgggcgagatggtcgagttcgagaacggcacgcgcggcatggcgctgaacctcgagctcgacaatgtcggcatcgtgatcttcggttccgaccgcgagatcaaggaaggccagaccgtcaagcggaccggcgccatcgtggacgcccccgtcggcaagggcctgctcggccgcgtcgtggacgctctcggcaacccgatcgacggcaagggcccgatcatgttcaccgagcgtcgccgggtcgacgtgaaggcgccgggcatcatcccgcgcaagtcggtgcacgagcccatgcagaccggcctgaaggccatcgatgcgctcatccccatcggccgcggccagcgcgagctcatcatcggcgaccgccagaccggcaagaccgccgtggcgctcgactcgatcctgaaccagaagcccatcaaccagggcgacgacgagaaggccaagctctactgcgtctatgtcgcggtgggccagaagcgttccactgtcgcgcagttcgtgaaggtgctcgaggagcacggcgcgctggaatattccatcgtcgtcgccgccaccgcctcggacgcggcccccatgcagttcctggcgccgttcaccggcaccgccatgggcgagtatttccgcgacaacggcatgcacgccctcatcatccatgatgacctgtccaagcaggccgtggcctaccgccagatgtcgctgctgctgcgccgcccgccgggccgcgaggcctatcccggcgatgtgttctacctgcactcccgcctcttggagcgcgccgccaagctcaatgacgagcacggcgccggctcgctgaccgccctgccggtgatcgagacccaggccaacgacgtgtcggcctacatcccgaccaacgtgatctccatcaccgacggtcagatcttccttgaatccgatctgttctaccagggcatccgcccggcggtgaacgtgggcctgtcggtgtcgcgcgtgggctcttcggcccagatcaaggcgatgaagcaggtggccggcaagatcaagggcgagctcgcccagtatcgcgagctggcggccttcgcccagttcggttcggacctggacgcggccacccagaagctgctgaaccgcggcgcccgcctcaccgagctgctgaagcagagccagttctcgcccctcaaggtggaggagcaggtggcggtgatctatgccggcaccaatggctatctcgatccgctgccggtctccaaggtgcgcgagttcgagcagggtctgctcctgtcgctgcgctcgcagcatccggagatcctggacgccatccgcacgtccaaggagctttccaaggacaccgccgagaagctgacgaaggccatcgacgccttcgccaagagcttctcctga

SEQ ID NO: 37 - protein, 509 aa, Unknown
  novel strain
MDIRAAEISAILKEQIQNFGQEAEVSEVGQVLSVGDGIARVYGLDNVQAGEMVEFENGTRGMALNLELDNVGIVIFGSDREIKEGQTVKRTGAIVDAPVGKGLLGRVVDALGNPIDGKGPIMFTERRRVDVKAPGIIPRKSVHEPMQTGLKAIDALIPIGRGQRELIIGDRQTGKTAVALDSILNQKPINQGDDEKAKLYCVYVAVGQKRSTVAQFVKVLEEHGALEYSIVVAATASDAAPMQFLAPFTGTAMGEYFRDNGMHALIIHDDLSKQAVAYRQMSLLLRRPPGREAYPGDVFYLHSRLLERAAKLNDEHGAGSLTALPVIETQANDVSAYIPTNVISITDGQIFLESDLFYQGIRPAVNVGLSVSRVGSSAQIKAMKQVAGKIKGELAQYRELAAFAQFGSDLDAATQKLLNRGARLTELLKQSQFSPLKVEEQVAVIYAGTNGYLDPLPVSKVREFEQGLLLSLRSQHPEILDAIRTSKELSKDTAEKLTKAIDAFAKSFS

SEQ ID NO: 38 - DNA, 555 bp, Unknown
  novel strain
gtggcggaaacgatcgtgtcaggcatggcgggacgctatgcgaccgcgctgttcgagctggcggacgaagccggtgccatcgattccgtccaggcggatcttgatcgcctgtccggccttctggccgagagcgcggatctggcgcggctggtcaagagcccggtcttcaccgccgagcagcagctcggcgcgatggcggccattctcgatcaagcaggcatttccggccttgcgggcaaattcgtgaagctggtggcgcagaaccgccgcctgttcgcactgccgcgcatgattgccgaatacgccgtcctggtggcccggaagaagggcgagacctcggcgagcgtgaccgttgccacccccctgagcgatgagcatctggccacgctcaaggcggccctggctgaaaagaccggcaaggacgtgaagctcgacgtcaccgtcgatccgtccatcctcggtggtctcatcgtgaagctcggctcgcgcatggtcgatgcttccctgaagaccaaactcaattctatccggcatgcgatgaaagaggtccgctga

SEQ ID NO: 39 - protein, 184 aa, Unknown
  novel strain
MAETIVSGMAGRYATALFELADEAGAIDSVQADLDRLSGLLAESADLARLVKSPVFTAEQQLGAMAAILDQAGISGLAGKFVKLVAQNRRLFALPRMIAEYAVLVARKKGETSASVTVATPLSDEHLATLKAALAEKTGKDVKLDVTVDPSILGGLIVKLGSRMVDASLKTKLNSIRHAMKEVR

SEQ ID NO: 40 - DNA, 492 bp, Unknown
  novel strain
atgaccgaaatggaactggctgagctctgggtcgccatcgccttcctggttttcgtaggcctcctgatctatgcgggcgcccaccgcgccatcgtctccgccctggattcccgcggctcgcgcatcgcctcggaactggaggaggcccgtcggctcaaggaagaggcccagaagctggtggccgaattcaagcgcaagcagcgcgaggccgaggccgaggccgaatccatcgtcaccggcgccaaggccgaggccgagcgcctcgccgccgaggccaaggcgaagatcgaggatttcgtcacccgccgcaccaagatggccgaggacaagatcgcccaggccgagcatcaggctctggcggacgtgaagtccatcgccgccgaggcggcggccaaggcggccgaggtgatcctcggcgcccaggccaccggcgcggtggcggagcgtctgctgtcgggcgccatctccgaggtcaagaccaagctcaactga

SEQ ID NO: 41 - protein, 163 aa, Unknown
  novel strain
MTEMELAELWVAIAFLVFVGLLIYAGAHRAIVSALDSRGSRIASELEEARRLKEEAQKLVAEFKRKQREAEAEAESIVTGAKAEAERLAAEAKAKIEDFVTRRTKMAEDKIAQAEHQALADVKSIAAEAAAKAAEVILGAQATGAVAERLLSGAISEVKTKLN

SEQ ID NO: 42 - DNA, 729 bp, Unknown
  novel strain
atgatgattgcatggaagcggaccttcgcagtcgtgaccttcggggccgccctgatggccatgcccgtcgcgggcgtggtcgcagctgagacttctcccgctccggcggcagtggcgcaggccgatcatgcggtgcccaccgaggcggccggccagggcaccgccgatgcggcccatgccgccgcgccgggcgaggccgcccatggtggcgcggccaagcacgaaacccatttcccgcccttcgacggcaccaccttcgcctcccagttgctgtggctcgccgtcaccttcggcctgctttactacctcatgagcaaggtcacgctgccgcgcatcggccgcatcctggaagagcgccacgaccgcatcgccgatgatctggaggaagcctccaagcatcgcgccgagagcgaggccgcccagcgggcctatgagaaggcgctgagcgaggcccgcgcgaaggcccattccatcgccgcggaaacccgcgaccgccttgccgcccacgccgacaccaaccgcaaggcgctggagagcgagctcaccgccaagctgcaggcggccgaggagcgcatcgccaccaccaagagcgaagccctcacccatgtgcgcggcatcgcggtggacgccacccaatccatcgtctccaccctcatcggtgtcgcgcccgcggcggccgacgtggaaaaagcggtggacggcgccctgtcccagcacggccaggcctga

SEQ ID NO: 43 - protein, 242 aa, Unknown
  novel strain
MMIAWKRTFAVVTFGAALMAMPVAGVVAAETSPAPAAVAQADHAVPTEAAGQGTADAAHAAAPGEAAHGGAAKHETHFPPFDGTTFASQLLWLAVTFGLLYYLMSKVTLPRIGRILEERHDRIADDLEEASKHRAESEAAQRAYEKALSEARAKAHSIAAETRDRLAAHADTNRKALESELTAKLQAAEERIATTKSEALTHVRGIAVDATQSIVSTLIGVAPAAADVEKAVDGALSQHGQA

SEQ ID NO: 44 - DNA, 228 bp, Unknown
  novel strain
atggaagcggaagctggaaagttcatcggtgccggcctcgcctgcctcggcatgggtctcgctggcgtcggcgtcggtaacatcttcggtaacttcctctccggcgccctgcgcaacccgtccgctgccgacggccagttcgcccgcgccttcatcggcgccgccctcgcggaaggtctcggcatcttctcgctggtcgttgcgctcgtcctgctgttcgtggcctga

SEQ ID NO: 45 - protein, 75 aa, Unknown
  novel strain
MEAEAGKFIGAGLACLGMGLAGVGVGNIFGNFLSGALRNPSAADGQFARAFIGAALAEGLGIFSLVVALVLLFVA

SEQ ID NO: 46 - DNA, 753 bp, Unknown
  novel strain
atgaccgtcgatccgatccaccagttcgagatcaagcgctacgtggatctgctgaacgtcggcggtgtccagttctccttcaccaacgcaacggtgttcatgattggcatcgtcctggtgattttcttcttcctgactttcgcgacacgcggtcgcacccttgtgccgggccggatgcagtcggcggcggagctgagctacgagttcatcgccaagatggtgcgcgacgcggccggcagcgagggaatggtgttctttcccttcgtcttctcgctcttcatgttcgtgctggtggcgaacgtattggggctcatcccctacaccttcacggtgaccgcccacctcatcgtcaccgccgccctggcggcgacggtgatcctcaccgtcatcatctacggcttcgtgcggcacggcacccacttcctgcacctgttcgtgccgtcgggcgtgccgggcttcctcctgcccttcctcgtggtgatcgaggtggtgtcgttcctgtcgcggcccatcagcctctcgctgcgtctgttcgccaacatgctggcgggccacatcgccctcaaggtgttcgccttcttcgtcgtgggactggcctcggccggcgcgatcggctggttcggcgccaccctgcccttcttcatgatcgtggcgctcaccgcgctggagctgctggtggcggtgctgcaggcctacgtgttcgcggtgctgacctcgatctacctcaacgacgccatccatcccggccactga

SEQ ID NO: 47 - protein, 250 aa, Unknown
  novel strain
MTVDPIHQFEIKRYVDLLNVGGVQFSFTNATVFMIGIVLVIFFFLTFATRGRTLVPGRMQSAAELSYEFIAKMVRDAAGSEGMVFFPFVFSLFMFVLVANVLGLIPYTFTVTAHLIVTAALAATVILTVIIYGFVRHGTHFLHLFVPSGVPGFLLPFLVVIEVVSFLSRPISLSLRLFANMLAGHIALKVFAFFVVGLASAGAIGWFGATLPFFMIVALTALELLVAVLQAYVFAVLTSIYLNDAIHPGH

SEQ ID NO: 48 - DNA, 390 bp, Unknown
  novel strain
atgtccgagccgaatgatccatcccgcagggacggtgcgaaggcgaaagacgagacgcaggactcccggcccggtgaggcggatcttgctcggcgcctcgatgcgctcggcacctccatcggtcaggtcaagtccagaagcggggagcccgcggcgacgccgcgcaaggacacctcctcggcctccggcgcggccctggcgtttcggctgggcgccgagtttgtttcaggcgtgctggtgggctcgctcatcggctacgggttggattatgcgtttgcgatttcgccctgggggctgatcgccttcacgctgatcggctttgccgccggcgtcctgaacatgctgcgcgtggcgaacagcgatgccaagcgccacagcgcggacaggtga

SEQ ID NO: 49 - protein, 129 aa, Unknown
  novel strain
MSEPNDPSRRDGAKAKDETQDSRPGEADLARRLDALGTSIGQVKSRSGEPAATPRKDTSSASGAALAFRLGAEFVSGVLVGSLIGYGLDYAFAISPWGLIAFTLIGFAAGVLNMLRVANSDAKRHSADR

SEQ ID NO: 50 - DNA, 1929 bp, Unknown
  novel strain
atgagttcgctctccgccactattcaacaggtcttcaacgagccgggctgcgcgaagaaccagaataagtccgaggcggagaagaagaagggctgcaccaagcagctgcaacccggcggagcggccggcggctgcgcgttcgacggcgcgaagatcgcgctccagcccttgaccgacgtcgcccacctggtgcacggccccatcgcctgcgaaggcaattcctgggacaatcgtggcgccaagtcctccggctcgaacatctggcgcaccggcttcaccacggacatcaacgaaaccgacgtggtgttcggcggcgagaagcgtctgttcaagtccatcaaggaaatcatcgagaagtacgacccgccggccgtcttcgtctatcagacctgcgtccccgccatgatcggcgacgacatcgacgcggtgtgcaaggcggccagggagaagttcggaaagccggtgatcccgatcaattcccccggcttcgtggggccgaagaatctcggcaacaagctcgccggcgaggcgctcctcgaccatgtgatcggcaccgaggagcccgattacacgacggcctacgacatcaacatcatcggcgaatacaatctctccggcgagttgtggcaggtgaagccgctgctggacgagctgggcatccgcatcctcgcctgcatctccggcgacgggaagtacaaggatgtggcgtcctcccaccgcgccaaggcggcgatgatggtgtgctccaaggccatgatcaacgtggcccgcaagatggaggagcgctacgacatccccttcttcgaaggctccttctacggcatcgaggatagctccgattccctgcgcgagattgcgcgcatgctcatcgagaagggcgccgatccggagctgatggaccgcaccgaggcgctgattgagcgggaagagaagaaggcgtgggacgccatcgccgcctacaagccccgcttcaaggacaagaaggtgctgctcatcaccggcggcgtgaaatcctggtcggtggtggcagcgctccaggaagccggcctcgaactggtgggcacctcggtgaagaagtccaccaaggaggacaaggagcgcatcaaggaactgatgggccaggacgcccacatgatcgacgacatgacgccccgcgaaatgtacaagatgctgaaggacgccaaggcggacatcatgctctcgggcgggcgctcgcaattcatcgcgctcaaggccgccatgccctggctcgacatcaaccaggagcgccaccacgcctatatgggctatgtgggcatggtgaagctggtcgaggagatcgacaaggcgctctacaatcccgtgtgggaacaggtgcgcaagcccgccccgtgggaaaatccggaagacacctggcaggcccgtgcgctcgccgaaatggaggcggaggccgccgcgctcgccgccgatccggtgcgcgcggaagaggtgcgccggtccaagaagatctgcaattgcaagagcgtcgacctcggaaccattgaggacgccatcaaggctcacgcgctgaccaccgtggagggtgtgcgagagcacaccaatgcctcgggaggctgcggagcctgcagcgggcggatcgaggagatcttcgaggccgtgggcgttgtcgccgccccgcctcccgcggaggccgccccgtctccgcaggagatcgcgcccgatccgctcgctgcggaggaaaagcgccgcgccaagaaggcctgcggctgcaaggaggtagcggtcggcaccattgaggatgccatccgcgccaagggtctgcgaaacatcgcggaggtgcgtgcggccaccgatgccaacaccggctgcggcaattgccaggagcgggtggagggcatcctcgaccgggttctcgccgaggcggcctcagaactccaggcggcggaatag

SEQ ID NO: 51 - protein, 642 aa, Unknown
  novel strain
MSSLSATIQQVFNEPGCAKNQNKSEAEKKKGCTKQLQPGGAAGGCAFDGAKIALQPLTDVAHLVHGPIACEGNSWDNRGAKSSGSNIWRTGFTTDINETDVVFGGEKRLFKSIKEIIEKYDPPAVFVYQTCVPAMIGDDIDAVCKAAREKFGKPVIPINSPGFVGPKNLGNKLAGEALLDHVIGTEEPDYTTAYDINIIGEYNLSGELWQVKPLLDELGIRILACISGDGKYKDVASSHRAKAAMMVCSKAMINVARKMEERYDIPFFEGSFYGIEDSSDSLREIARMLIEKGADPELMDRTEALIEREEKKAWDAIAAYKPRFKDKKVLLITGGVKSWSVVAALQEAGLELVGTSVKKSTKEDKERIKELMGQDAHMIDDMTPREMYKMLKDAKADIMLSGGRSQFIALKAAMPWLDINQERHHAYMGYVGMVKLVEEIDKALYNPVWEQVRKPAPWENPEDTWQARALAEMEAEAAALAADPVRAEEVRRSKKICNCKSVDLGTIEDAIKAHALTTVEGVREHTNASGGCGACSGRIEEIFEAVGVVAAPPPAEAAPSPQEIAPDPLAAEEKRRAKKACGCKEVAVGTIEDAIRAKGLRNIAEVRAATDANTGCGNCQERVEGILDRVLAEAASELQAAE

SEQ ID NO: 52 - DNA, 1503 bp, Unknown
  novel strain
atgagtgtcgcacagtcccagagcgtcgccgagatcaaggcgcgcaacaaggaactcatcgaagaggtcctcaaggtctatcccgagaagaccgccaagcgccgcgccaagcacctgaacgtccacgaagccggcaagtccgactgcggcgtgaagtccaacatcaagtccatcccgggcgtgatgaccatccgcggttgcgcttatgccggctccaagggtgtggtgtggggtcccatcaaggacatgatccacatctcccacggcccggtgggctgcggccagtatagctgggccgcccgccgcaactactatatcggcacgaccggcatcgacaccttcgtgacgatgcagttcacctccgacttccaggagaaggacatcgtcttcggcggcgacaagaagctcgccaagatcatggacgagatccaggagctgttcccgctgaacaacggcatcaccgttcagtccgagtgccccatcggcctcatcggcgacgacatcgaggccgtctccaagcagaagtccaaggagtatgagggcaagaccatcgtgccggtgcgctgcgagggcttccgcggcgtgtcccagtccctgggccaccacatcgccaacgacgccatccgcgattgggtgttcgacaagatcgcgcccgacgccgagccgcgctttgagccgaccccgtacgacgtcgccatcatcggcgactacaatatcggtggtgacgcctggtcgtcccgtatcctcctggaggagatgggcctgcgcgtgatcgcccagtggtccggcgacggttcgctcgctgagctggaggccaccccgaaggccaagctcaacgtgctgcactgctaccgctccatgaactacatctcgcgccacatggaagagaagtacggtatcccgtggtgcgagtacaacttcttcggtccttccaagatcgccgagtccctgcgcaagatcgccagctacttcgacgacaagatcaaggaaggcgcggagcgcgtcatcgccaagtatcagccgctcatggatgcggtgatcgcgaagtatcgtccccgcctcgagggcaagaccgtgatgctgtacgtgggcggcctgcgtccccgtcacgtcatcggcgcctacgaggacctgggcatggaagtggtcggcacgggctacgagttcgcccataacgacgactaccagcgcaccgcccagcactacgtcaaggatggcaccatcatctatgacgacgtgaccggctacgagttcgagaagttcgtcgagaagatccagccggacctggtcggttcgggcatcaaggaaaagtacgtcttccagaagatgggcgtgccgttccgccagatgcactcctgggactactcgggcccgtaccacggctatgacggcttcgcgatcttcgcgcgcgacatggacatggccatcaacagccccgtgtggaagatgacccaggctccgtggaagagcgtccccaagccgacgatgctcgcggctgaatga

SEQ ID NO: 53 - protein, 500 aa, Unknown
  novel strain
MSVAQSQSVAEIKARNKELIEEVLKVYPEKTAKRRAKHLNVHEAGKSDCGVKSNIKSIPGVMTIRGCAYAGSKGVVWGPIKDMIHISHGPVGCGQYSWAARRNYYIGTTGIDTFVTMQFTSDFQEKDIVFGGDKKLAKIMDEIQELFPLNNGITVQSECPIGLIGDDIEAVSKQKSKEYEGKTIVPVRCEGFRGVSQSLGHHIANDAIRDWVFDKIAPDAEPRFEPTPYDVAIIGDYNIGGDAWSSRILLEEMGLRVIAQWSGDGSLAELEATPKAKLNVLHCYRSMNYISRHMEEKYGIPWCEYNFFGPSKIAESLRKIASYFDDKIKEGAERVIAKYQPLMDAVIAKYRPRLEGKTVMLYVGGLRPRHVIGAYEDLGMEVVGTGYEFAHNDDYQRTAQHYVKDGTIIYDDVTGYEFEKFVEKIQPDLVGSGIKEKYVFQKMGVPFRQMHSWDYSGPYHGYDGFAIFARDMDMAINSPVWKMTQAPWKSVPKPTMLAAE

SEQ ID NO: 54 - DNA, 1377 bp, Unknown
  novel strain
atggccaccgtttccgtctccaagaaggcctgcgcggtcaaccccctcaagatgagccagccggtgggcggcgcgctcgccttcatgggcgtgcgcaaggccatgccgctgctgcacggctcgcagggctgcacctccttcggcctggtgctgttcgtgcgccacttcaaggaagccatccccatgcagaccaccgccatgagcgaggtggcgacggttctgggcggccttgagaatgtggagcaggccattctcaacatctacaatcgcaccaagccggagatcatcggcatctgctccaccggcgtcaccgagaccaagggcgatgatgtcgacggctacatcaagctgatccgggacaagtatccccagctggccgacttcccgctggtctatgtctccacccccgatttcaaggacgccttccaggacggttgggagaagaccgtggcgaagatggtggaggcgctggtgaagcccgccgccgacaagcagaaggacaagacccgcgtcaacgtcctgcccggctgccacctcacgcccggcgatctggatgagatgcggaccatcttcgaggatttcgggctcacaccctatttcctgccggatctggccggctcgctggatgggcatatccccgaggacttctcgcccaccaccatcggcggcatcggcatcgatgagatcgccaccatgggcgaggcggcccacaccatctgcatcggcgcgcagatgcgccgggcgggcgaggccatggagaagaagaccggcattcccttcaagctgttcgagcgcctgtgcggcctggaggcgaacgacgccttcatcatgcacctgtcgcagatctccggccggccggtgccggtgaagtatcgccggcagcggggccagctggtggatgccatgctggacggccacttccatctgggcggtcgcaaggtggccatgggggcggagccggacctgctctacgacgtgggctccttcctgcacgagatgggcgcccacatcctttccgcggtcaccaccacccagtcgccggtgctggcgcgcctgcctgccgaggaggtgcttatcggcgacctggaggatctggagacccaggcgaaggcgcgcggatgcgatctcctgctcacccattcccatgggcgccaggcggcggagcgcctccacatccccttctaccggatcggcattcccatgtttgaccggctgggggcggggcatctgttgtcggtgggctatcgcggcacccgcgacctcatcttccatctcgccaaccttgtgatcgccgaccacgaggaaaatcacgagccgacgcccgacacctgggccaccggccatggcgagcatgccgccgcccccacttcccattga

SEQ ID NO: 55 - protein, 458 aa, Unknown
  novel strain
MATVSVSKKACAVNPLKMSQPVGGALAFMGVRKAMPLLHGSQGCTSFGLVLFVRHFKEAIPMQTTAMSEVATVLGGLENVEQAILNIYNRTKPEIIGICSTGVTETKGDDVDGYIKLIRDKYPQLADFPLVYVSTPDFKDAFQDGWEKTVAKMVEALVKPAADKQKDKTRVNVLPGCHLTPGDLDEMRTIFEDFGLTPYFLPDLAGSLDGHIPEDFSPTTIGGIGIDEIATMGEAAHTICIGAQMRRAGEAMEKKTGIPFKLFERLCGLEANDAFIMHLSQISGRPVPVKYRRQRGQLVDAMLDGHFHLGGRKVAMGAEPDLLYDVGSFLHEMGAHILSAVTTTQSPVLARLPAEEVLIGDLEDLETQAKARGCDLLLTHSHGRQAAERLHIPFYRIGIPMFDRLGAGHLLSVGYRGTRDLIFHLANLVIADHEENHEPTPDTWATGHGEHAAAPTSH

SEQ ID NO: 56 - DNA, 1560 bp, Unknown
  novel strain
atgccacaaaatgctgacaatgtgctcgatcacttcgagctcttccgtggtcccgaataccagcagatgctggccaataagaaaaagatgttcgagaacccccgcgatccggccgaagtcgagcgcgtgcgggaatgggcgaagactcctgaatacaaggagctgaacttcgcccgcgaggcgctcaccgtgaatccggccaaggcttgtcagccgctgggcgcggtgttcgtcgccgtcggcttcgagagcacgatccccttcgtgcacggctcgcagggttgcgtcgcgtattaccgctcgcacctctcccgccacttcaaggagccgtcctcctgcgtctcctcgtccatgaccgaggatgcggcggtgttcggcggcctcaacaacatgattgacggcctcgccaacacctacaacatgtacaagccgaagatgatcgccgtctccaccacctgcatggcggaagtcatcggcgacgatctgaacgccttcatcaagaccgcgaaggaaaagggctcggttccggccgaatacgacgtgcccttcgcccacaccccggcgttcgtcggcagccatgtcaccggctacgacaatgcgctcaagggcatcctcgagcacttctgggacggcaaggccggcaccgcgccgaagctggagcgcgttcccaacgagaagatcaacttcatcggcggcttcgacggctacaccgtcggcaacactcgcgaagtgaagcgcatcttcgaggcgttcggcgccgattacaccatcctcgccgacaattccgaagtgttcgacaccccgaccgacggcgagttccgcatgtatgacggcggcacgaccctggaggacgcggcgaacgcggtgcacgccaaggccaccatctccatgcaggaatactgcacggagaagaccctgcccatgatcgccggtcatggccaggacgtggtcgccctcaaccaccccgtgggcgtgggcggcaccgacaagttcctcatggagatcgcccgcctcaccggcaaggagatccccgaggagctgacccgcgagcgcggccgtctcgtggacgctatcgcggactcttccgcgcacatccacggcaagaagttcgccatctacggcgatccggatctgtgcctgggcctcgccgcgttcctgctggagctgggcgccgagccgacccatgtgctggccaccaacggcaccaagaagtgggccgagaaggttcaggaactgttcgactcttcgccgttcggcgccaactgcaaggtctatcccggcaaggacctgtggcacatgcgctcgctcctgttcgtggagccggtggatttcatcatcggcaacacctacggcaagtatctcgagcgcgacacgggcaccccgctgatccgtatcggcttcccggtgttcgaccgtcaccaccaccaccgccgtccggtgtggggctatcagggcggcatgaacgtcctgatcacgatcctcgacaagatctttgacgagatcgaccgcaacaccaacgtgccggccaagaccgactactcgttcgacatcattcgttga

SEQ ID NO: 57 - protein, 519 aa, Unknown
  novel strain
MPQNADNVLDHFELFRGPEYQQMLANKKKMFENPRDPAEVERVREWAKTPEYKELNFAREALTVNPAKACQPLGAVFVAVGFESTIPFVHGSQGCVAYYRSHLSRHFKEPSSCVSSSMTEDAAVFGGLNNMIDGLANTYNMYKPKMIAVSTTCMAEVIGDDLNAFIKTAKEKGSVPAEYDVPFAHTPAFVGSHVTGYDNALKGILEHFWDGKAGTAPKLERVPNEKINFIGGFDGYTVGNTREVKRIFEAFGADYTILADNSEVFDTPTDGEFRMYDGGTTLEDAANAVHAKATISMQEYCTEKTLPMIAGHGQDVVALNHPVGVGGTDKFLMEIARLTGKEIPEELTRERGRLVDAIADSSAHIHGKKFAIYGDPDLCLGLAAFLLELGAEPTHVLATNGTKKWAEKVQELFDSSPFGANCKVYPGKDLWHMRSLLFVEPVDFIIGNTYGKYLERDTGTPLIRIGFPVFDRHHHHRRPVWGYQGGMNVLITILDKIFDEIDRNTNVPAKTDYSFDIIR

SEQ ID NO: 58 - DNA, 621 bp, Unknown
  novel strain
gtggagtccggtggtcctgagccgggcgtgggctgcgccggccgcggcgtgatcacctccatcaacttcctggaggagaacggcgcctacgaggacatcgactatgtgtcctacgacgtgctgggcgacgtggtgtgcggcggcttcgccatgcccatccgcgagaacaaggcgcaggaaatctacatcgtgatgtccggcgagatgatggccatgtatgcggccaacaacatctccaagggcatcctgaagtatgccaattccggcggcgtgcgcctgggcgggctggtctgcaacgagcgccagaccgacaaggagctggagctggcggaggctctggcgaagaagctcggcaccgagctgatctacttcgtgccgcgcgacaacatcgtgcagcatgccgagctgcgccgcatgacagtgatcgagtatgcgcccgattccgcccaggcccagcactaccggaacctggccgagaaggtgcacgccaacaagggcaacggcatcatcccgaccccgatcaccatggacgagctggaagacatgctcatggagcacggcatcatgaaggccgtggacgagagccagatcggcaagaccgccgccgagctcgccgtctga

SEQ ID NO: 59 - protein, 206 aa, Unknown
  novel strain
MESGGPEPGVGCAGRGVITSINFLEENGAYEDIDYVSYDVLGDVVCGGFAMPIRENKAQEIYIVMSGEMMAMYAANNISKGILKYANSGGVRLGGLVCNERQTDKELELAEALAKKLGTELIYFVPRDNIVQHAELRRMTVIEYAPDSAQAQHYRNLAEKVHANKGNGIIPTPITMDELEDMLMEHGIMKAVDESQIGKTAAELAV